European Patent Specification EP 2 967 015 B9, published August 9, 2023. Title: Genetically Modified Major Histocompatibility Complex Animals. Applicant: Lynn Macdonald Andrew J Murphy Naxin Tu Cagan Gurer Vera Voronina Sean Stevens. Application TBA. The sequence listing filed with the application follows.

SEQUENCE LISTING (40 sequences)

SEQ ID NO: 1 - DNA, 19 bp, Artificial Sequence
  Synthetic
cagaacgccaggctgtaac

SEQ ID NO: 2 - DNA, 20 bp, Artificial Sequence
  Synthetic
ggagagcagggtcagtcaac

SEQ ID NO: 3 - DNA, 24 bp, Artificial Sequence
  Synthetic
caccgccactcacagctccttaca

SEQ ID NO: 4 - DNA, 22 bp, Artificial Sequence
  Synthetic
gtgggcaccatcttcatcattc

SEQ ID NO: 5 - DNA, 22 bp, Artificial Sequence
  Synthetic
cttcctttccagggtgtgactc

SEQ ID NO: 6 - DNA, 23 bp, Artificial Sequence
  Synthetic
aggcctgcgatcaggtggcacct

SEQ ID NO: 7 - DNA, 17 bp, Artificial Sequence
  Synthetic
tgcggccgatcttagcc

SEQ ID NO: 8 - DNA, 18 bp, Artificial Sequence
  Synthetic
ttgaccgattccttgcgg

SEQ ID NO: 9 - DNA, 21 bp, Artificial Sequence
  Synthetic
acgagcgggttcggcccattc

SEQ ID NO: 10 - DNA, 140 bp, Artificial Sequence
  Synthetic
tttgtaaacaaagtctacccagagacagatgacagacttcagctccaatgctgattggttcctcacttgggaccaaccctctcgagtaccgttcgtataatgtatgctatacgaagttatatgcatccgggtaggggagg

SEQ ID NO: 11 - DNA, 140 bp, Artificial Sequence
  Synthetic
cctcgacctgcagccctaggataacttcgtataatgtatgctatacgaacggtagagctccacaggcatttgggtgggcagggatggacggtgactgggacaatcgggatggaagagcatagaatgggagttagggaaga

SEQ ID NO: 12 - DNA, 110 bp, Artificial Sequence
  Synthetic
tgctgattggttcctcacttgggaccaaccctaagctttatctatgtcgggtgcggagaaagaggtaatgaaatggcacaaggagatcacacacccaaaccaaactcgcc

SEQ ID NO: 13 - DNA, 96 bp, Artificial Sequence
  Synthetic
cacatcagtgaggctagaataaattaaaatcgctaatatgaaaatggggatttgtacctctgagtgtgaaggctgggaagactgctttcaagggac

SEQ ID NO: 14 - DNA, 150 bp, Artificial Sequence
  Synthetic
tccatcacttcactgggtagcacagctgtaactgtccagcctgggtaccgagctcggatccactagtaacggccgccagtgtgctggaattcgcccttgatcgagctccctgggctgcaggtggtgggcgttgcgggtggggccggttaa

SEQ ID NO: 15 - DNA, 80 bp, Artificial Sequence
  Synthetic
atctccatcagaagggcaccggtataacttcgtataaggtatcctatacgaagttatatgcatggcctccgcgccgggtt

SEQ ID NO: 16 - DNA, 90 bp, Artificial Sequence
  Synthetic
ataacttcgtataaggtatcctatacgaagttatctcgagtggcttacaggtaggtgcgtgaagcttctacaagcacagttgccccctgg

SEQ ID NO: 17 - DNA, 90 bp, Artificial Sequence
  Synthetic
ctgtttcttccctaactcccattctatgctcttccatcccgaccgcggcccaatctctctccactacttcctgcctacatgtatgtaggt

SEQ ID NO: 18 - DNA, 80 bp, Artificial Sequence
  Synthetic
caaggtttcctcctatgatgcttgtgtgaaactcggggccggccagcatttaacagtacagggatgggagcacagctcac

SEQ ID NO: 19 - DNA, 80 bp, Artificial Sequence
  Synthetic
gaaagcagtcttcccagccttcacactcagaggtacaaatccccattttcatattagcgattttaatttattctagcctc

SEQ ID NO: 20 - DNA, 80 bp, Artificial Sequence
  Synthetic
tcttccctaactcccattctatgctcttccatcccgaccgcggcccaatctctctccactacttcctgcctacatgtatg

SEQ ID NO: 21 - DNA, 21 bp, Artificial Sequence
  Synthetic
ctggcggcttgaagaatttgg

SEQ ID NO: 22 - DNA, 24 bp, Artificial Sequence
  Synthetic
catgatttccaggttggctttgtc

SEQ ID NO: 23 - DNA, 26 bp, Artificial Sequence
  Synthetic
cgatttgccagctttgaggctcaagg

SEQ ID NO: 24 - DNA, 20 bp, Artificial Sequence
  Synthetic
aggcttgggtgctccacttg

SEQ ID NO: 25 - DNA, 21 bp, Artificial Sequence
  Synthetic
gaccctggtgatgctggaaac

SEQ ID NO: 26 - DNA, 27 bp, Artificial Sequence
  Synthetic
caggtgtaaacctctccactccgagga

SEQ ID NO: 27 - DNA, 100 bp, Artificial Sequence
  Synthetic
gaagagactgcccggcccgaggccccgaggcccgacggtccccagagagcgtggtcgcgcgggctgttccacagctccgggccgggtcagggtggcggct

SEQ ID NO: 28 - DNA, 100 bp, Artificial Sequence
  Synthetic
agagctccttctgacccatcccttcccatctcttatccctgatgtcactgaccggtataacttcgtataatgtatgctatacgaagttatatgcatggcc

SEQ ID NO: 29 - DNA, 100 bp, Artificial Sequence
  Synthetic
cgccataacttcgtataatgtatgctatacgaagttatgtcgacctcgagctatatgatctgcttccactactgagctgagacctacaggaaatcatatc

SEQ ID NO: 30 - DNA, 100 bp, Artificial Sequence
  Synthetic
gtgggttgggcttatggaatgacatgaaatctagctttaggagctttttagaagtgtggaaaacaagttttgggatataggagtaaaaggcaggaagttc

SEQ ID NO: 31 - DNA, 159 bp, Artificial Sequence
  Synthetic
ccttaatacacaaaatgatgaaagaaactgactttcaaatattacgggctctcgagcggccgccagtgtgatggatggtacctaactataacggtcctaaggtagcgaccattttttggggtttgtttctaccactcattcctccctcccacttggtat

SEQ ID NO: 32 - DNA, 280 bp, Artificial Sequence
  Synthetic
cccaattcccaatttcttccttccctcactgggcccactagtagaatcatggtttggtggattgtgagctgacggccggcccaaccagagcctcctgaagaatggatcacacagttgttagacctcttcatattgagaatttgtatctccctcttctgtgggtttcccattgcccggctccaggcatccctcagctgcacaactcacccacaatgtcttcacctccacagaggctgagcatggtggtcagggcgaggacccccagaatcagagctctgct

SEQ ID NO: 33 - DNA, 100 bp, Artificial Sequence
  Synthetic
cggctgctgtggtggtgctgatggtgctgagcagcccagggactgagggcagagactctcccggtaagtgcagggccactgctctccagagccgccactc

SEQ ID NO: 34 - DNA, 100 bp, Artificial Sequence
  Synthetic
gagctccttctgacccattccttcccatctcttatccctgatgtcactacctcgagataacttcgtataatgtatgctatacgaagttatatgcatggcc

SEQ ID NO: 35 - DNA, 100 bp, Artificial Sequence
  Synthetic
tacgaagttatacgcgtaactataacggtcctaaggtagcgagcggccgcctatatgatctgcttccactactgagctgagacctacaggaaatcatatc

SEQ ID NO: 36 - DNA, 136 bp, Artificial Sequence
  Synthetic
agggtgagggggcaagttaatctacatagcctttgtgggttgggcttatgggcgcgccattcgctaccttaggaccgttatagttatgaagtgtggaaaacaagttttgggatatagagtaaaaggcaggaagttc

SEQ ID NO: 37 - DNA, 100 bp, Artificial Sequence
  Synthetic
ttcagctccagagaacattcctcactcatgcactcacccacaatgtcttcacctccacagaggctgagcatggtggtcagggcgaggacccccagaatca

SEQ ID NO: 38 - DNA, 100 bp, Artificial Sequence
  Synthetic
gagttcctccatcacttcactgggtagcacagctgtaactgtccagcctgtcctgggctgcaggtggtgggcgttgcgggtggggccggttaaggttcca

SEQ ID NO: 39 - DNA, 100 bp, Artificial Sequence
  Synthetic
tcccacatcctattttaatttgctccatgttctcatctccatcagcacagctcgagataacttcgtataatgtatgctatacgaagttatatgcatggcc

SEQ ID NO: 40 - DNA, 100 bp, Artificial Sequence
  Synthetic
atacgaagttatgctagtaactataacggtcctaaggtagcgagtggcttacaggtaggtgcgtgaagcttctacaagcacagttgccccctgggaagca